European Patent Specification EP 3 835 430 B1, published August 16, 2023. Title: COMPOSITIONS AND METHODS FOR THE DETECTION AND ANALYSIS OF MYCOBACTERIUM TUBERCULOSIS. Applicant: ABBOTT MOLECULAR INC. Application PCT/US2015/039362. The sequence listing filed with the application follows.

SEQUENCE LISTING (36 sequences)

SEQ ID NO: 1 - DNA, 23 bp, Artificial Sequence
  Synthetic
cctgcgagcgtaggcgtcggtga

SEQ ID NO: 2 - DNA, 22 bp, Artificial Sequence
  Synthetic
cgtccagcgccgcttcggacca

SEQ ID NO: 3 - DNA, 27 bp, Artificial Sequence
  Synthetic
gcacctcaagctgaacggaaaagtcct

SEQ ID NO: 4 - DNA, 22 bp, Artificial Sequence
  Synthetic
ccggggttgagcgcagcgatct

SEQ ID NO: 5 - DNA, 20 bp, Artificial Sequence
  Synthetic
  misc_feature (1)..(1): 5' propynyl Du
  misc_feature (5)..(5): 5' propynyl Du
  misc_feature (10)..(10): 5' propynyl Du
  misc_feature (11)..(11): 5' propynyl dC
  misc_feature (12)..(12): 5' propynyl Du
  misc_feature (14)..(14): 5' propynyl dC
  misc_feature (15)..(15): 5' propynyl Du
  misc_feature (17)..(19): 5' propynyl dC
naggngaggnnngnnannnt

SEQ ID NO: 6 - DNA, 19 bp, Artificial Sequence
  Synthetic
  misc_feature (1)..(1): 5' propynyl Du
  misc_feature (3)..(4): 5' propynyl dC
  misc_feature (9)..(9): 5' propynyl dC
  misc_feature (11)..(12): 5' propynyl dC
  misc_feature (14)..(14): 5' propynyl Du
  misc_feature (15)..(15): 5' propynyl dC
nannagggnannannaaat

SEQ ID NO: 7 - DNA, 28 bp, Artificial Sequence
  Synthetic
ctacagcagagttggcagcttcactttc

SEQ ID NO: 8 - DNA, 22 bp, Artificial Sequence
  Synthetic
gtctggcctttcagcaagtttc

SEQ ID NO: 9 - DNA, 19 bp, Artificial Sequence
  Synthetic
  misc_feature (3)..(3): 5' propynyl dC
  misc_feature (7)..(8): 5' propynyl Du
  misc_feature (9)..(9): 5' propynyl dC
  misc_feature (11)..(11): 5' propynyl Du
  misc_feature (17)..(17): 5' propynyl dC
gangagnnnangagggnat

SEQ ID NO: 10 - DNA, 26 bp, Artificial Sequence
  Synthetic
gccgcttcggaccaccagcacctaac

SEQ ID NO: 11 - DNA, 28 bp, Artificial Sequence
  Synthetic
gtaggcgtcggtgacaaaggccacgtag

SEQ ID NO: 12 - DNA, 18 bp, Artificial Sequence
  Synthetic
tgcccaggtcgacacata

SEQ ID NO: 13 - DNA, 25 bp, Artificial Sequence
  Synthetic
tacgaccacatcaaccgggagccca

SEQ ID NO: 14 - DNA, 25 bp, Artificial Sequence
  Synthetic
gcgtggacgcggctgatgtgctcct

SEQ ID NO: 15 - DNA, 17 bp, Artificial Sequence
  Synthetic
ccgcgagctgcgcgatg

SEQ ID NO: 16 - DNA, 28 bp, Artificial Sequence
  Synthetic
gcacgctgctctacccgctgttcaacct

SEQ ID NO: 17 - DNA, 26 bp, Artificial Sequence
  Synthetic
gtgccctgagcggtgatcgtgacgtt

SEQ ID NO: 18 - DNA, 17 bp, Artificial Sequence
  Synthetic
tccggcctttcacgaga

SEQ ID NO: 19 - DNA, 20 bp, Artificial Sequence
  Synthetic
tcggggctcgggtagaagtt

SEQ ID NO: 20 - DNA, 20 bp, Artificial Sequence
  Synthetic
tcgtcaactcgggcagcaac

SEQ ID NO: 21 - DNA, 17 bp, Artificial Sequence
  Synthetic
tactcggctcacgcacg

SEQ ID NO: 22 - DNA, 24 bp, Artificial Sequence
  Synthetic
ggctcgggtagaagttcgacttgg

SEQ ID NO: 23 - DNA, 21 bp, Artificial Sequence
  Synthetic
gtcaactcgggcagcaacgac

SEQ ID NO: 24 - DNA, 19 bp, Artificial Sequence
  Synthetic
ctcacgcacggcggtattc

SEQ ID NO: 25 - DNA, 17 bp, Artificial Sequence
  Synthetic
ggcagcggactcgggtt

SEQ ID NO: 26 - DNA, 18 bp, Artificial Sequence
  Synthetic
accgcagttcgggctctc

SEQ ID NO: 27 - DNA, 17 bp, Artificial Sequence
  Synthetic
tcacgacgacgagcgac

SEQ ID NO: 28 - DNA, 23 bp, Artificial Sequence
  Synthetic
cgctgatgaccagtgtgttgatt

SEQ ID NO: 29 - DNA, 22 bp, Artificial Sequence
  Synthetic
gcagcatcagatcgagcaggac

SEQ ID NO: 30 - DNA, 17 bp, Artificial Sequence
  Synthetic
atggtccggcagctctc

SEQ ID NO: 31 - DNA, 26 bp, Artificial Sequence
  Synthetic
caacatcagcctgcccagttactacc

SEQ ID NO: 32 - DNA, 21 bp, Artificial Sequence
  Synthetic
cttcgcgtggagtggacgatg

SEQ ID NO: 33 - DNA, 20 bp, Artificial Sequence
  Synthetic
aagtcgctggaaaattacat

SEQ ID NO: 34 - DNA, 27 bp, Artificial Sequence
  Synthetic
cgtggaggcgatcacaccgcagacgtt

SEQ ID NO: 35 - DNA, 26 bp, Artificial Sequence
  Synthetic
cgttgatcaacatccggccggtggtc

SEQ ID NO: 36 - DNA, 21 bp, Artificial Sequence
  Synthetic
cggtctgtcacgtgagcgtgc